European Patent Specification EP 3 570 814 B1, published November 29, 2023. Title: MOLECULAR ADJUVANTS FOR ENHANCED CYTOSOLIC DELIVERY OF ACTIVE AGENTS. Applicant: Universiteit Gent. The sequence listing filed with the application follows.

SEQUENCE LISTING (16 sequences)

SEQ ID NO: 1 - RNA, 21 nt, Artificial Sequence
  siRNA - Sense
ugcgcuacgaucgacgaugtt

SEQ ID NO: 2 - RNA, 21 nt, Artificial Sequence
  siRNA - Antisense
caucgucgaucguagcgcatt

SEQ ID NO: 3 - RNA, 21 nt, Artificial Sequence
  siRNA - Sense
ugcgcuacgaucgacgaugtt

SEQ ID NO: 4 - RNA, 21 nt, Artificial Sequence
  siRNA - Antisense
caucgucgaucguagcgcatt

SEQ ID NO: 5 - RNA, 21 nt, Artificial Sequence
  siRNA - Sense
uagcgacuaaacacaucaauu

SEQ ID NO: 6 - RNA, 21 nt, Artificial Sequence
  siRNA - Antisense
uugauguguuuagucgcuauu

SEQ ID NO: 7 - RNA, 21 nt, Artificial Sequence
  siRNA - Sense
caagcugacccugaaguuctt

SEQ ID NO: 8 - RNA, 21 nt, Artificial Sequence
  siRNA - Antisense
gaacuucagggucagcuugtt

SEQ ID NO: 9 - RNA, 21 nt, Artificial Sequence
  siRNA - Sense
caagcugacccugaaguucuu

SEQ ID NO: 10 - RNA, 21 nt, Artificial Sequence
  siRNA - Antisense
gaacuucagggucagcuuguu

SEQ ID NO: 11 - RNA, 21 nt, Artificial Sequence
  siRNA - Sense
caaccaaagucgaauaugauu

SEQ ID NO: 12 - RNA, 21 nt, Artificial Sequence
  siRNA - Antisense
ucauauucgacuuugguuguu

SEQ ID NO: 13 - RNA, 23 nt, Artificial Sequence
  DsiRNA - Sense
acccugaaguucaucugcaccac

SEQ ID NO: 14 - RNA, 27 nt, Artificial Sequence
  DsiRNA - Antisense
acugggacuucaaguagacgugguggc

SEQ ID NO: 15 - RNA, 25 nt, Artificial Sequence
  DsiRNA - Sense
gguuccuggaacaauugcuuuuaca

SEQ ID NO: 16 - RNA, 27 nt, Artificial Sequence
  DsiRNA - Antisense
gaccaaggaccuuguuaacgaaaaugu